European Patent Specification EP 3 247 328 B1, published January 7, 2026. Title: METHODS, COMPOSITIONS, AND SYSTEMS FOR DELIVERING THERAPEUTIC AND DIAGNOSTIC AGENTS INTO CELLS. Applicant: PhaseRx, Inc. The sequence listing filed with the application follows.

SEQUENCE LISTING (51 sequences)

SEQ ID NO: 1 - protein, 354 aa, Homo sapiens
  TRANSIT (1)..(34): native mitochondrial leader seqeuence
MLFNLRILLNNAAFRNGHNFMVRNFRCGQPLQNKVQLKGRDLLTLKNFTGEEIKYMLWLSADLKFRIKQKGEYLPLLQGKSLGMIFEKRSTRTRLSTETGFALLGGHPCFLTTQDIHLGVNESLTDTARVLSSMADAVLARVYKQSDLDTLAKEASIPIINGLSDLYHPIQILADYLTLQEHYSSLKGLTLSWIGDGNNILHSIMMSAAKFGMHLQAATPKGYEPDASVTKLAEQYAKENGTKLLLTNDPLEAAHGGNVLITDTWISMGQEEEKKKRLQAFQGYQVTMKTAKVAASDWTFLHCLPRKPEEVDDEVFYSPRSLVFPEAENRKWTIMAVMVSLLTDYSPQLQKPKF

SEQ ID NO: 2 - protein, 354 aa, Artificial
  Human ornithine transcarbamylase with mouse mitochondrial leader sequence
  TRANSIT (1)..(34): mouse mitochondrial leader sequence
MLSNLRILLNNAALRKGHTSVVRHFWCGKPVQSQVQLKGRDLLTLKNFTGEEIKYMLWLSADLKFRIKQKGEYLPLLQGKSLGMIFEKRSTRTRLSTETGFALLGGHPCFLTTQDIHLGVNESLTDTARVLSSMADAVLARVYKQSDLDTLAKEASIPIINGLSDLYHPIQILADYLTLQEHYSSLKGLTLSWIGDGNNILHSIMMSAAKFGMHLQAATPKGYEPDASVTKLAEQYAKENGTKLLLTNDPLEAAHGGNVLITDTWISMGQEEEKKKRLQAFQGYQVTMKTAKVAASDWTFLHCLPRKPEEVDDEVFYSPRSLVFPEAENRKWTIMAVMVSLLTDYSPQLQKPKF

SEQ ID NO: 3 - DNA, 1262 bp, Artificial
  cDNA encoding human ornithine transcarbamylase, codon-optimized for mouse expression
  promoter (1)..(20): T7 promoter
taatacgactcactatagggaaataagagagaaaagaagagtaagaagaaatataagagccaccatgctgttcaacctcagaatcctcctcaataacgccgcctttagaaacggtcataacttcatggtcagaaactttagatgtggtcagcctctccagaacaaagtgcagctcaaggggcgggacctgctcaccctgaaaaatttcacaggcgaggaaatcaagtacatgctctggctgtctgccgatctgaagttcaggatcaagcagaagggcgaatatctcccactgctccaggggaaaagtctgggtatgatcttcgaaaagcggagtactaggaccagactgtcaacagagactggattcgctctgctcggaggacacccatgctttctgaccacacaggacattcatctcggtgtgaacgagtcactgaccgacacagctcgagtcctcagctccatggcagatgccgtgctggcaagggtctacaaacagagtgacctcgataccctggctaaggaagcaagcatccccatcattaatggactctccgacctgtatcaccctatccagattctggccgattacctcaccctgcaggagcattattctagtctgaaagggctcacactgagctggattggcgacggaaacaatatcctgcactccattatgatgtctgccgctaagtttggcatgcatctgcaggcagccacaccaaaaggatacgaacccgatgcttccgtgactaagctggccgaacagtatgctaaagagaacggaactaagctgctcctgaccaatgaccccctggaggctgcacacgggggtaacgtcctgatcactgatacctggatttccatgggccaggaggaagagaagaaaaagcgcctgcaggcattccagggataccaggtgacaatgaaaactgccaaggtcgccgcttctgattggacttttctccattgtctgccccgaaagcctgaagaggtggacgatgaggtcttctattcacctcggagcctggtgtttccagaagccgagaatcgcaagtggacaatcatggcagtgatggtgtccctcctcacagactattccccacagctccagaagcccaagttttgagcggccgcttaattaagctgccttctgcggggcttgccttctggccatgcccttcttctctcccttgcacctgtacctcttggtctttgaataaagcctgagtaggaagtctagagtttaaacatttaaatct

SEQ ID NO: 4 - DNA, 1262 bp, Artificial
  cDNA encoding human ornithine transcarbamylase with mouse mitochondrial leader sequence, codon-optimized for mouse expression
  promoter (1)..(20): T7 promoter
taatacgactcactatagggaaataagagagaaaagaagagtaagaagaaatataagagccaccatgctctctaacctcaggattctgctcaacaacgctgctctgcggaaaggccatacctctgtcgtcaggcacttctggtgtgggaaacccgtgcagagccaggtgcagctcaaggggcgggacctgctcaccctgaaaaatttcacaggcgaggaaatcaagtacatgctctggctgtctgccgatctgaagttcaggatcaagcagaagggcgaatatctcccactgctccaggggaaaagtctgggtatgatcttcgaaaagcggagtactaggaccagactgtcaacagagactggattcgctctgctcggaggacacccatgctttctgaccacacaggacattcatctcggtgtgaacgagtcactgaccgacacagctcgagtcctcagctccatggcagatgccgtgctggcaagggtctacaaacagagtgacctcgataccctggctaaggaagcaagcatccccatcattaatggactctccgacctgtatcaccctatccagattctggccgattacctcaccctgcaggagcattattctagtctgaaagggctcacactgagctggattggcgacggaaacaatatcctgcactccattatgatgtctgccgctaagtttggcatgcatctgcaggcagccacaccaaaaggatacgaacccgatgcttccgtgactaagctggccgaacagtatgctaaagagaacggaactaagctgctcctgaccaatgaccccctggaggctgcacacgggggtaacgtcctgatcactgatacctggatttccatgggccaggaggaagagaagaaaaagcgcctgcaggcattccagggataccaggtgacaatgaaaactgccaaggtcgccgcttctgattggacttttctccattgtctgccccgaaagcctgaagaggtggacgatgaggtcttctattcacctcggagcctggtgtttccagaagccgagaatcgcaagtggacaatcatggcagtgatggtgtccctcctcacagactattccccacagctccagaagcccaagttttgagcggccgcttaattaagctgccttctgcggggcttgccttctggccatgcccttcttctctcccttgcacctgtacctcttggtctttgaataaagcctgagtaggaagtctagagtttaaacatttaaatct

SEQ ID NO: 5 - DNA, 1262 bp, Artificial
  cDNA encoding human ornithine transcarbamylase, codon-optimized for human expression
  promoter (1)..(20): T7 promoter
taatacgactcactatagggaaataagagagaaaagaagagtaagaagaaatataagagccaccatgctgtttaacctgaggattctgctgaacaacgctgcttttcggaacggccacaactttatggtgcggaactttcggtgcggacagccactgcagaacaaagtgcagctgaaggggagggacctgctgaccctgaaaaatttcacaggagaggaaatcaagtacatgctgtggctgtctgccgatctgaagttccggatcaagcagaagggcgaatatctgccactgctgcagggcaaaagtctggggatgatcttcgaaaagaggagtactcggaccagactgtcaacagagactggattcgctctgctgggaggacacccatgctttctgaccacacaggacattcatctgggcgtgaacgagtcactgaccgacacagctcgagtcctgagctccatggcagatgccgtgctggcacgggtctacaaacagagcgacctggataccctggctaaggaagcaagcatccccatcattaatgggctgtccgacctgtatcaccctatccagattctggccgattacctgaccctgcaggagcattattctagtctgaaaggcctgacactgagctggattggggacggaaacaatatcctgcactccattatgatgtctgccgctaagtttggaatgcatctgcaggcagccacaccaaaaggctacgaacccgatgccagtgtgactaagctggccgaacagtatgctaaagagaacggcactaagctgctgctgaccaatgaccctctggaggctgcacacggaggcaacgtcctgatcactgatacctggatttccatgggccaggaggaagagaagaaaaagcgcctgcaggcattccaggggtaccaggtgacaatgaaaactgccaaggtcgccgcttctgattggacttttctgcattgtctgccccgaaaacctgaagaggtggacgatgaggtcttctattcacctaggagcctggtgtttccagaagccgagaatcgcaagtggacaatcatggctgtgatggtgtccctgctgactgattattccccccagctgcagaaacctaagttctgagcggccgcttaattaagctgccttctgcggggcttgccttctggccatgcccttcttctctcccttgcacctgtacctcttggtctttgaataaagcctgagtaggaagtctagagtttaaacatttaaatct

SEQ ID NO: 6 - RNA, 1221 nt, Artificial
  mRNA encoding human ornithine transcarbamylase, codon-optimized for mouse expression
gggaaauaagagagaaaagaagaguaagaagaaauauaagagccaccaugcuguucaaccucagaauccuccucaauaacgccgccuuuagaaacggucauaacuucauggucagaaacuuuagauguggucagccucuccagaacaaagugcagcucaaggggcgggaccugcucacccugaaaaauuucacaggcgaggaaaucaaguacaugcucuggcugucugccgaucugaaguucaggaucaagcagaagggcgaauaucucccacugcuccaggggaaaagucuggguaugaucuucgaaaagcggaguacuaggaccagacugucaacagagacuggauucgcucugcucggaggacacccaugcuuucugaccacacaggacauucaucucggugugaacgagucacugaccgacacagcucgaguccucagcuccauggcagaugccgugcuggcaagggucuacaaacagagugaccucgauacccuggcuaaggaagcaagcauccccaucauuaauggacucuccgaccuguaucacccuauccagauucuggccgauuaccucacccugcaggagcauuauucuagucugaaagggcucacacugagcuggauuggcgacggaaacaauauccugcacuccauuaugaugucugccgcuaaguuuggcaugcaucugcaggcagccacaccaaaaggauacgaacccgaugcuuccgugacuaagcuggccgaacaguaugcuaaagagaacggaacuaagcugcuccugaccaaugacccccuggaggcugcacacggggguaacguccugaucacugauaccuggauuuccaugggccaggaggaagagaagaaaaagcgccugcaggcauuccagggauaccaggugacaaugaaaacugccaaggucgccgcuucugauuggacuuuucuccauugucugccccgaaagccugaagagguggacgaugaggucuucuauucaccucggagccugguguuuccagaagccgagaaucgcaaguggacaaucauggcagugauggugucccuccucacagacuauuccccacagcuccagaagcccaaguuuugagcggccgcuuaauuaagcugccuucugcggggcuugccuucuggccaugcccuucuucucucccuugcaccuguaccucuuggucuuugaauaaagccugaguaggaag

SEQ ID NO: 7 - RNA, 1221 nt, Artificial
  mRNA encoding human ornithine transcarbamylase with mouse mitochondrial leader sequence, codon-optimized for mouse expression
gggaaauaagagagaaaagaagaguaagaagaaauauaagagccaccaugcucucuaaccucaggauucugcucaacaacgcugcucugcggaaaggccauaccucugucgucaggcacuucuggugugggaaacccgugcagagccaggugcagcucaaggggcgggaccugcucacccugaaaaauuucacaggcgaggaaaucaaguacaugcucuggcugucugccgaucugaaguucaggaucaagcagaagggcgaauaucucccacugcuccaggggaaaagucuggguaugaucuucgaaaagcggaguacuaggaccagacugucaacagagacuggauucgcucugcucggaggacacccaugcuuucugaccacacaggacauucaucucggugugaacgagucacugaccgacacagcucgaguccucagcuccauggcagaugccgugcuggcaagggucuacaaacagagugaccucgauacccuggcuaaggaagcaagcauccccaucauuaauggacucuccgaccuguaucacccuauccagauucuggccgauuaccucacccugcaggagcauuauucuagucugaaagggcucacacugagcuggauuggcgacggaaacaauauccugcacuccauuaugaugucugccgcuaaguuuggcaugcaucugcaggcagccacaccaaaaggauacgaacccgaugcuuccgugacuaagcuggccgaacaguaugcuaaagagaacggaacuaagcugcuccugaccaaugacccccuggaggcugcacacggggguaacguccugaucacugauaccuggauuuccaugggccaggaggaagagaagaaaaagcgccugcaggcauuccagggauaccaggugacaaugaaaacugccaaggucgccgcuucugauuggacuuuucuccauugucugccccgaaagccugaagagguggacgaugaggucuucuauucaccucggagccugguguuuccagaagccgagaaucgcaaguggacaaucauggcagugauggugucccuccucacagacuauuccccacagcuccagaagcccaaguuuugagcggccgcuuaauuaagcugccuucugcggggcuugccuucuggccaugcccuucuucucucccuugcaccuguaccucuuggucuuugaauaaagccugaguaggaag

SEQ ID NO: 8 - RNA, 1221 nt, Artificial
  mRNA encoding human ornithine transcarbamylase, codon-optimized for human expression
gggaaauaagagagaaaagaagaguaagaagaaauauaagagccaccaugcuguuuaaccugaggauucugcugaacaacgcugcuuuucggaacggccacaacuuuauggugcggaacuuucggugcggacagccacugcagaacaaagugcagcugaaggggagggaccugcugacccugaaaaauuucacaggagaggaaaucaaguacaugcuguggcugucugccgaucugaaguuccggaucaagcagaagggcgaauaucugccacugcugcagggcaaaagucuggggaugaucuucgaaaagaggaguacucggaccagacugucaacagagacuggauucgcucugcugggaggacacccaugcuuucugaccacacaggacauucaucugggcgugaacgagucacugaccgacacagcucgaguccugagcuccauggcagaugccgugcuggcacgggucuacaaacagagcgaccuggauacccuggcuaaggaagcaagcauccccaucauuaaugggcuguccgaccuguaucacccuauccagauucuggccgauuaccugacccugcaggagcauuauucuagucugaaaggccugacacugagcuggauuggggacggaaacaauauccugcacuccauuaugaugucugccgcuaaguuuggaaugcaucugcaggcagccacaccaaaaggcuacgaacccgaugccagugugacuaagcuggccgaacaguaugcuaaagagaacggcacuaagcugcugcugaccaaugacccucuggaggcugcacacggaggcaacguccugaucacugauaccuggauuuccaugggccaggaggaagagaagaaaaagcgccugcaggcauuccagggguaccaggugacaaugaaaacugccaaggucgccgcuucugauuggacuuuucugcauugucugccccgaaaaccugaagagguggacgaugaggucuucuauucaccuaggagccugguguuuccagaagccgagaaucgcaaguggacaaucauggcugugauggugucccugcugacugauuauuccccccagcugcagaaaccuaaguucugagcggccgcuuaauuaagcugccuucugcggggcuugccuucuggccaugcccuucuucucucccuugcaccuguaccucuuggucuuugaauaaagccugaguaggaag

SEQ ID NO: 9 - protein, 750 aa, Homo sapiens
  TRANSIT (1)..(32): native mitochondrial leader sequence
MLRAKNQLFLLSPHYLRQVKESSGSRLIQQRLLHQQQPLHPEWAALAKKQLKGKNPEDLIWHTPEGISIKPLYSKRDTMDLPEELPGVKPFTRGPYPTMYTFRPWTIRQYAGFSTVEESNKFYKDNIKAGQQGLSVAFDLATHRGYDSDNPRVRGDVGMAGVAIDTVEDTKILFDGIPLEKMSVSMTMNGAVIPVLANFIVTGEEQGVPKEKLTGTIQNDILKEFMVRNTYIFPPEPSMKIIADIFEYTAKHMPKFNSISISGYHMQEAGADAILELAYTLADGLEYSRTGLQAGLTIDEFAPRLSFFWGIGMNFYMEIAKMRAGRRLWAHLIEKMFQPKNSKSLLLRAHCQTSGWSLTEQDPYNNIVRTAIEAMAAVFGGTQSLHTNSFDEALGLPTVKSARIARNTQIIIQEESGIPKVADPWGGSYMMECLTNDVYDAALKLINEIEEMGGMAKAVAEGIPKLRIEECAARRQARIDSGSEVIVGVNKYQLEKEDAVEVLAIDNTSVRNRQIEKLKKIKSSRDQALAERCLAALTECAASGDGNILALAVDASRARCTVGEITDALKKVFGEHKANDRMVSGAYRQEFGESKEITSAIKRVHKFMEREGRRPRLLVAKMGQDGHDRGAKVIATGFADLGFDVDIGPLFQTPREVAQQAVDADVHAVGISTLAAGHKTLVPELIKELNSLGRPDILVMCGGVIPPQDYEFLFEVGVSNVFGPGTRIPKAAVQVLDDIEKCLEKKQQSV

SEQ ID NO: 10 - RNA, 2409 nt, Artificial
  mRNA encoding human methylmalonyl-coenzyme A mutase
gggaaauaagagagaaaagaagaguaagaagaaauauaagagccaccauguuaagagcuaagaaucagcuuuuuuuacuuucaccucauuaccugaggcagguaaaagaaucaucaggcuccaggcucauacagcaacgacuucuacaccagcaacagccccuucacccagaaugggcugcccuggcuaaaaagcagcugaaaggcaaaaacccagaagaccuaauauggcacaccccggaagggaucucuauaaaacccuuguauuccaagagagauacuauggacuuaccugaagaacuuccaggagugaagccauucacacguggaccauauccuaccauguauaccuuuaggcccuggaccauccgccaguaugcugguuuuaguacuguggaagaaagcaauaaguucuauaaggacaacauuaaggcuggucagcagggauuaucaguugccuuugaucuggcgacacaucguggcuaugauucagacaacccucgaguucguggugauguuggaauggcuggaguugcuauugacacuguggaagauaccaaaauucuuuuugauggaauuccuuuagaaaaaaugucaguuuccaugacuaugaauggagcaguuauuccaguucuugcaaauuuuauaguaacuggagaagaacaagguguaccuaaagagaagcuuacugguaccauccaaaaugauauacuaaaggaauuuaugguucgaaauacauacauuuuuccuccagaaccauccaugaaaauuauugcugacauauuugaauauacagcaaagcacaugccaaaauuuaauucaauuucaauuaguggauaccauaugcaggaagcaggggcugaugccauucuggagcuggccuauacuuuagcagauggauuggaguacucuagaacuggacuccaggcuggccugacaauugaugaauuugcaccaagguugucuuucuucuggggaauuggaaugaauuucuauauggaaauagcaaagaugagagcugguagaagacucugggcucacuuaauagagaaaauguuucagccuaaaaacucaaaaucucuucuucuaagagcacacugucagacaucuggauggucacuuacugagcaggaucccuacaauaauauuguccguacugcaauagaagcaauggcagcaguauuuggagggacucagucuuugcacacaaauucuuuugaugaagcuuuggguuugccaacugugaaaagugcucgaauugccaggaacacacaaaucaucauucaagaagaaucugggauucccaaaguggcugauccuuggggagguucuuacaugauggaaugucucacaaaugauguuuaugaugcugcuuuaaagcucauuaaugaaauugaagaaauggguggaauggccaaagcuguagcugagggaauaccuaaacuucgaauugaagaaugugcugcccgaagacaagcuagaauagauucugguucugaaguaauuguuggaguaaauaaguaccaguuggaaaaagaagacgcuguagaaguucuggcaauugauaauacuucagugcgaaacaggcagauugaaaaacuuaagaagaucaaauccagcagggaucaagcuuuggcugaacguugucuugcugcacuaaccgaaugugcugcuagcggagauggaaauauccuggcucuugcaguggaugcaucucgggcaagauguacagugggagaaaucacagaugcccugaaaaagguauuuggugaacauaaagcgaaugaucgaauggugaguggagcauaucgccaggaauuuggagaaaguaaagagauaacaucugcuaucaagaggguucauaaauucauggaacgugaaggucgcagaccucgucuucuuguagcaaaaaugggacaagauggccaugacagaggagcaaaaguuauugcuacaggauuugcugaucuugguuuugauguggacauaggcccucuuuuccagacuccucgugaaguggcccagcaggcuguggaugcggaugugcaugcugugggcauaagcacccucgcugcuggucauaaaacccuaguuccugaacucaucaaagaacuuaacucccuuggacggccagauauucuugucauguguggaggggugauaccaccucaggauuaugaauuucuguuugaaguugguguuuccaauguauuugguccugggacucgaauuccaaaggcugccguucaggugcuugaugauauugagaaguguuuggaaaagaagcagcaaucuguauaagcggccgcuuaauuaagcugccuucugcggggcuugccuucuggccaugcccuucuucucucccuugcaccuguaccucuuggucuuugaauaaagccugaguaggaag

SEQ ID NO: 11 - protein, 728 aa, Homo sapiens
  TRANSIT (1)..(52): native mitochondrial leader sequence
MAGFWVGTAPLVAAGRRGRWPPQQLMLSAALRTLKHVLYYSRQCLMVSRNLGSVGYDPNEKTFDKILVANRGEIACRVIRTCKKMGIKTVAIHSDVDASSVHVKMADEAVCVGPAPTSKSYLNMDAIMEAIKKTRAQAVHPGYGFLSENKEFARCLAAEDVVFIGPDTHAIQAMGDKIESKLLAKKAEVNTIPGFDGVVKDAEEAVRIAREIGYPVMIKASAGGGGKGMRIAWDDEETRDGFRLSSQEAASSFGDDRLLIEKFIDNPRHIEIQVLGDKHGNALWLNERECSIQRRNQKVVEEAPSIFLDAETRRAMGEQAVALARAVKYSSAGTVEFLVDSKKNFYFLEMNTRLQVEHPVTECITGLDLVQEMIRVAKGYPLRHKQADIRINGWAVECRVYAEDPYKSFGLPSIGRLSQYQEPLHLPGVRVDSGIQPGSDISIYYDPMISKLITYGSDRTEALKRMADALDNYVIRGVTHNIALLREVIINSRFVKGDISTKFLSDVYPDGFKGHMLTKSEKNQLLAIASSLFVAFQLRAQHFQENSRMPVIKPDIANWELSVKLHDKVHTVVASNNGSVFSVEVDGSKLNVTSTWNLASPLLSVSVDGTQRTVQCLSREAGGNMSIQFLGTVYKVNILTRLAAELNKFMLEKVTEDTSSVLRSPMPGVVVAVSVKPGDAVAEGQEICVIEAMKMQNSMTAGKTGTVKSVHCQAGDTVGEGDLLVELE

SEQ ID NO: 12 - RNA, 2343 nt, Artificial
  mRNA encoding human propionyl CoA carboxylase, alpha polypeptide (PCCA)
gggaaauaagagagaaaagaagaguaagaagaaauauaagagccaccauggcgggguucugggucgggacagcaccgcuggucgcugccggacggcgugggcgguggccgccgcagcagcugaugcugagcgcggcgcugcggacccugaagcauguucuguacuauucaagacagugcuuaauggugucccguaaucuugguucagugggauaugauccuaaugaaaaaacuuuugauaaaauucuuguugcuaauagaggagaaauugcaugucggguuauuagaacuugcaagaagaugggcauuaagacaguugccauccacagugauguugaugcuaguucuguucaugugaaaauggcggaugaggcugucuguguuggcccagcucccaccaguaaaagcuaccucaacauggaugccaucauggaagccauuaagaaaaccagggcccaagcuguacauccagguuauggauuccuuucagaaaacaaagaauuugccagauguuuggcagcagaagaugucguuuucauuggaccugacacacaugcuauucaagccaugggcgacaagauugaaagcaaauuauuagcuaagaaagcagagguuaauacaaucccuggcuuugauggaguagucaaggaugcagaagaagcugucagaauugcaagggaaauuggcuacccugucaugaucaaggccucagcaggugguggugggaaaggcaugcgcauugcuugggaugaugaagagaccagggaugguuuuagauugucaucucaagaagcugcuucuaguuuuggcgaugauagacuacuaauagaaaaauuuauugauaauccucgucauauagaaauccagguucuaggugauaaacaugggaaugcuuuauggcuuaaugaaagagagugcucaauucagagaagaaaucagaaggugguggaggaagcaccaagcauuuuuuuggaugcggagacucgaagagcgaugggagaacaagcuguagcucuugccagagcaguaaaauauuccucugcugggaccguggaguuccuuguggacucuaagaagaauuuuuauuucuuggaaaugaauacaagacuccagguugagcauccugucacagaaugcauuacuggccuggaccuaguccaggaaaugauccguguugcuaagggcuacccucucaggcacaaacaagcugauauucgcaucaacggcugggcaguugaaugucggguuuaugcugaggaccccuacaagucuuuugguuuaccaucuauugggagauugucucaguaccaagaaccguuacaucuaccugguguccgaguggacaguggcauccaaccaggaagugauauuagcauuuauuaugauccuaugauuucaaaacuaaucacauauggcucugauagaacugaggcacugaagagaauggcagaugcacuggauaacuauguuauucgagguguuacacauaauauugcauuacuucgagaggugauaaucaacucacgcuuuguaaaaggagacaucagcacuaaauuucucuccgauguguauccugauggcuucaaaggacacaugcuaaccaagagugagaagaaccaguuauuggcaauagcaucaucauuguuuguggcauuccaguuaagagcacaacauuuucaagaaaauucaagaaugccuguuauuaaaccagacauagccaacugggagcucucaguaaaauugcaugauaaaguucauaccguaguagcaucaaacaaugggucaguguucucgguggaaguugaugggucgaaacuaaaugugaccagcacguggaaccuggcuucgcccuuauugucugucagcguugauggcacucagaggacuguccagugucuuucucgagaagcagguggaaacaugagcauucaguuucuugguacaguguacaaggugaauaucuuaaccagacuugccgcagaauugaacaaauuuaugcuggaaaaagugacugaggacacaagcaguguucugcguuccccgaugcccggaguggugguggccgucucugucaagccuggagacgcgguagcagaaggucaagaaauuugugugauugaagccaugaaaaugcagaauaguaugacagcugggaaaacuggcacggugaaaucugugcacugucaagcuggagacacaguuggagaaggggaucugcucguggagcuggaaugagcggccgcuuaauuaagcugccuucugcggggcuugccuucuggccaugcccuucuucucucccuugcaccuguaccucuuggucuuugaauaaagccugaguaggaag

SEQ ID NO: 13 - protein, 539 aa, Homo sapiens
  TRANSIT (1)..(28): native mitochondrial leader sequence
MAAALRVAAVGARLSVLASGLRAAVRSLCSQATSVNERIENKRRTALLGGGQRRIDAQHKRGKLTARERISLLLDPGSFVESDMFVEHRCADFGMAADKNKFPGDSVVTGRGRINGRLVYVFSQDFTVFGGSLSGAHAQKICKIMDQAITVGAPVIGLNDSGGARIQEGVESLAGYADIFLRNVTASGVIPQISLIMGPCAGGAVYSPALTDFTFMVKDTSYLFITGPDVVKSVTNEDVTQEELGGAKTHTTMSGVAHRAFENDVDALCNLRDFFNYLPLSSQDPAPVRECHDPSDRLVPELDTIVPLESTKAYNMVDIIHSVVDEREFFEIMPNYAKNIIVGFARMNGRTVGIVGNQPKVASGCLDINSSVKGARFVRFCDAFNIPLITFVDVPGFLPGTAQEYGGIIRHGAKLLYAFAEATVPKVTVITRKAYGGAYDVMSSKHLCGDTNYAWPTAEIAVMGAKGAVEIIFKGHENVEAAQAEYIEKFANPFPAAVRGFVDDIIQPSSTRARICCDLDVLASKKVQRPWRKHANIPL

SEQ ID NO: 14 - RNA, 1776 nt, Artificial
  mRNA encoding human propionyl CoA carboxylase, beta polypeptide (PCCB)
gggaaauaagagagaaaagaagaguaagaagaaauauaagagccaccauggcggcggcauuacggguggcggcggucggggcaaggcucagcguucuggcgagcggucuccgcgccgcgguccgcagccuuugcagccaggccaccucuguuaacgaacgcaucgaaaacaagcgccggaccgcgcugcugggagggggccaacgccguauugacgcgcagcacaagcgaggaaagcuaacagccagggagaggaucagucucuugcuggacccuggcagcuuuguugagagcgacauguuuguggaacacagaugugcagauuuuggaauggcugcugauaagaauaaguuuccuggagacagcguggucacuggacgaggccgaaucaauggaagauugguuuaugucuucagucaggauuuuacaguuuuuggaggcagucugucaggagcacaugcccaaaagaucugcaaaaucauggaccaggccauaacggugggggcuccagugauugggcugaaugacucugggggagcacggauccaagaaggaguggagucuuuggcuggcuaugcagacaucuuucugaggaauguuacggcauccggagucaucccucagauuucucugaucaugggcccaugugcugguggggccgucuacuccccagcccuaacagacuucacguucaugguaaaggacaccuccuaccuguucaucacuggcccugauguugugaagucugucaccaaugaggauguuacccaggaggagcucgguggugccaagacccacaccaccaugucagguguggcccacagagcuuuugaaaaugauguugaugccuuguguaaucuccgggauuucuucaacuaccugccccugagcagucaggacccggcucccguccgugagugccacgaucccagugaccgucugguuccugagcuugacacaauugucccuuuggaaucaaccaaagccuacaacaugguggacaucauacacucuguuguugaugagcgugaauuuuuugagaucaugcccaauuaugccaagaacaucauuguugguuuugcaagaaugaaugggaggacuguuggaauuguuggcaaccaaccuaagguggccucaggaugcuuggauauuaauucaucugugaaaggggcucguuuugucagauucugugaugcauucaauauuccacucaucacuuuuguugaugucccuggcuuucuaccuggcacagcacaggaauacgggggcaucauccggcauggugccaagcuucucuacgcauuugcugaggcaacuguacccaaagucacagucaucaccaggaaggccuauggaggugccuaugaugucaugagcucuaagcaccuuuguggugauaccaacuaugccuggcccaccgcagagauugcagucaugggagcaaagggcgcuguggagaucaucuucaaagggcaugagaauguggaagcugcucaggcagaguacaucgagaaguuugccaacccuuucccugcagcagugcgaggguuuguggaugacaucauccaaccuucuuccacacgugcccgaaucugcugugaccuggaugucuuggccagcaagaagguacaacguccuuggagaaaacaugcaaauauuccauuguaagcggccgcuuaauuaagcugccuucugcggggcuugccuucuggccaugcccuucuucucucccuugcaccuguaccucuuggucuuugaauaaagccugaguaggaag

SEQ ID NO: 15 - protein, 30 aa, Artificial
  GALA peptide
WEAALAEALAEALAEHLAEALAEALEALAA

SEQ ID NO: 16 - protein, 18 aa, Artificial
  truncated GALA peptide
CAEALAEALAEALAEALA

SEQ ID NO: 17 - protein, 26 aa, Apis mellifera
GIGAVLKVLTTGLPALISWIKRKRQQ

SEQ ID NO: 18 - protein, 27 aa, Artificial
  Melittin peptide with N-terminal cysteine
CGIGAVLKVLTTGLPALISWIKRKRQQ

SEQ ID NO: 19 - protein, 21 aa, Artificial
  HPH-1 peptide
FIIDIIAFLLMGGFIVYVKNL

SEQ ID NO: 20 - protein, 24 aa, Artificial
  HPH-1 peptide with N-terminal Cys-Ala-Ala
CAAFIIDIIAFLLMGGFIVYVKNL

SEQ ID NO: 21 - protein, 17 aa, Artificial
  sHGP peptide
CARGWEVLKYWWNLLQY

SEQ ID NO: 22 - protein, 30 aa, Artificial
  bPrPp peptide
MVKSKIGSWILVLFVAMWSDVGLCKKRPKP

SEQ ID NO: 23 - protein, 18 aa, Artificial
  MAP peptide
KLALKLALKALKAALKLA

SEQ ID NO: 24 - protein, 11 aa, Artificial
  PTD4 peptide
YARAAARQARA

SEQ ID NO: 25 - protein, 29 aa, Artificial
  Maurocalcine peptide
GDCLPHLKLCKENKDCCSKKCKRRGTNIE

SEQ ID NO: 26 - protein, 10 aa, Artificial
  SynB3 peptide
RRLSYSRRRF

SEQ ID NO: 27 - protein, 18 aa, Artificial
  SynB1 peptide
RGGRLSYSRRRFSTSTGR

SEQ ID NO: 28 - protein, 17 aa, Artificial
  YTA4 peptide
IAWVKAFIRKLRKGPLG

SEQ ID NO: 29 - protein, 16 aa, Artificial
  YTA2 peptide
YTAIAWVKAFIRKLRK

SEQ ID NO: 30 - protein, 20 aa, Artificial
  CADY peptide
GLWRALWRLLRSLWRLLWRA

SEQ ID NO: 31 - protein, 15 aa, Artificial
  Pep-3 peptide
KWFETWFTEWPKKRK

SEQ ID NO: 32 - protein, 21 aa, Artificial
  Pep-1 peptide
KETWWETWWTEWSQPKKKRKV

SEQ ID NO: 33 - protein, 21 aa, Artificial
  PepFect peptide (amide linkage from epsilon amino group of Lys7)
AGYLLGKINLKALAALAKKIL

SEQ ID NO: 34 - protein, 21 aa, Artificial
  PepFect-3 peptide
AGYLLGKINLKALAALAKKIL

SEQ ID NO: 35 - protein, 16 aa, Artificial
  Penetratin peptide
RQIKIWFQNRRMKWKK

SEQ ID NO: 36 - protein, 30 aa, Artificial
  KALA peptide
WEAKLAKALAKALAKHLAKALAKALKACEA

SEQ ID NO: 37 - protein, 18 aa, Artificial
  pVEC peptide
LLIILRRRIRKQAHAHSK

SEQ ID NO: 38 - protein, 29 aa, Artificial
  RVG peptide
YTIWMPENPRPGTPCDIFTNSRGKRASNG

SEQ ID NO: 39 - protein, 16 aa, Artificial
  MPS peptide
AAVALLPAVLLALLAK

SEQ ID NO: 40 - protein, 27 aa, Artificial
  Transportan peptide
GWTLNSAGYLLGKINLKALAALAKKIL

SEQ ID NO: 41 - protein, 12 aa, Artificial
  TAT peptide
GRKKRRQRRPPQ

SEQ ID NO: 42 - protein, 20 aa, Artificial
  BMV Gag-(7-25) peptide
KMTRAQRRAAARRNRRWTAR

SEQ ID NO: 43 - protein, 28 aa, Artificial
  hCT(18-32)-k7 peptide (branched structure between Ala13 and Lys14)
KKRKAPKKKRKFAKFHTFPQTAIGVGAP

SEQ ID NO: 44 - protein, 22 aa, Artificial
  M1073 peptide
MVTVLFRRLRIRRASGPPRVRV

SEQ ID NO: 45 - protein, 23 aa, Artificial
  EB1 peptide
LIRLWSHLIHIWFQNRRLKWKKK

SEQ ID NO: 46 - protein, 27 aa, Artificial
  MPG-beta peptide
GALFLGFLGAAGSTMGAWSQPKKKRKV

SEQ ID NO: 47 - protein, 27 aa, Artificial
  MPG-beta peptide
GALFLAFLAAALSLMGLWSQPKKKRKV

SEQ ID NO: 48 - protein, 464 aa, Homo sapiens
MASESGKLWGGRFVGAVDPIMEKFNASIAYDRHLWEVDVQGSKAYSRGLEKAGLLTKAEMDQILHGLDKVAEEWAQGTFKLNSNDEDIHTANERRLKELIGATAGKLHTGRSRNDQVVTDLRLWMRQTCSTLSGLLWELIRTMVDRAEAERDVLFPGYTHLQRAQPIRWSHWILSHAVALTRDSERLLEVRKRINVLPLGSGAIAGNPLGVDRELLRAELNFGAITLNSMDATSERDFVAEFLFWASLCMTHLSRMAEDLILYCTKEFSFVQLSDAYSTGSSLMPQKKNPDSLELIRSKAGRVFGRCAGLLMTLKGLPSTYNKDLQEDKEAVFEVSDTMSAVLQVATGVISTLQIHQENMGQALSPDMLATDLAYYLVRKGMPFRQAHEASGKAVFMAETKGVALNQLSLQELQTISPLFSGDVICVWDYGHSVEQYGALGGTARSSVDWQIRQVRALLQAQQA

SEQ ID NO: 49 - RNA, 1551 nt, Artificial
  mRNA encoding human argininosuccinate lyase (ASL) isoform 1, codon-optimized for mouse expression
gggaaauaagagagaaaagaagaguaagaagaaauauaagagccaccauggcaucagagagcgguaaacuguggggugggagauucgugggugccgucgauccuauuauggagaaauucaacgccagcauugccuacgacagacaccugugggagguggacguccagggcucaaaggccuacagccggggucuggagaaggcaggccugcucacaaaagccgaaauggaccagauccugcacggacucgauaagguggcugaggaaugggcacaggggacauucaaacugaacucuaacgacgaggauauccacacugcuaacgagaggagacugaaggaacucauuggcgccacagcuggaaaacugcauacuggacggagccgcaacgaccagguggucacagaucugagacucuggaugcggcagaccugcucuacacugaguggacugcucugggagcucauucgaacuaugguggacagggcagaggccgaaagagacguccuguuuccaggauauacccaccugcagcgagcacagccaaucagguggucucacuggauucugagucacgcuguggcacucacccgcgauucugagcgacugcucgaagugcgaaagaggaucaacguccugccucucgggaguggugccauugcugggaauccacuggguguggacagggagcugcucagagcugaacugaacuucggcgcaaucacccugaauucaauggacgccacaagcgagcgcgauuuugucgccgaauuccucuuuugggcuagucugugcaugacccaucucucaaggauggcugaggaccugauccucuacuguacaaaggaauucagcuuugugcagcuguccgacgcauauucuacugguagcucccugaugccccagaagaaaaacccugacucccuggagcucauuagaucuaaggcaggacgaguguucggaaggugcgcagggcugcucaugacucugaaaggccucccauccaccuacaauaaggaccugcaggaggauaaagaagccguguuugaagucagugacacaaugucagcugugcugcaggucgcaacuggugugaucagcacccugcagauucaccaggaaaacaugggacaggcucuguccccagacaugcuggccacugaucucgcuuacuaucuggugcgaaagggaaugccuuucaggcaggcacacgaggccagcggcaaggcaguguuuauggccgaaaccaaaggcgucgcccugaaucagcugucccuccaggagcugcagacaaucagcccccucuucuccggggacgugauuugugucugggauuacggacacucuguggaacaguacggggcccugggcggaaccgcuagaagcagcgucgauuggcagauuaggcagguccgagcccuccuccaggcacagcaggccugagcggccgcuuaauuaagcugccuucugcggggcuugccuucuggccaugcccuucuucucucccuugcaccuguaccucuuggucuuugaauaaagccugaguaggaag

SEQ ID NO: 50 - protein, 412 aa, Homo sapiens
MSSKGSVVLAYSGGLDTSCILVWLKEQGYDVIAYLANIGQKEDFEEARKKALKLGAKKVFIEDVSREFVEEFIWPAIQSSALYEDRYLLGTSLARPCIARKQVEIAQREGAKYVSHGATGKGNDQVRFELSCYSLAPQIKVIAPWRMPEFYNRFKGRNDLMEYAKQHGIPIPVTPKNPWSMDENLMHISYEAGILENPKNQAPPGLYTKTQDPAKAPNTPDILEIEFKKGVPVKVTNVKDGTTHQTSLELFMYLNEVAGKHGVGRIDIVENRFIGMKSRGIYETPAGTILYHAHLDIEAFTMDREVRKIKQGLGLKFAELVYTGFWHSPECEFVRHCIAKSQERVEGKVQVSVLKGQVYILGRESPLSLYNEELVSMNVQGDYEPTDATGFININSLRLKEYHRLQSKVTAK

SEQ ID NO: 51 - RNA, 1395 nt, Artificial
  mRNA encoding human argininosuccinate synthetase (ASS1), codon-optimized for mouse expression
gggaaauaagagagaaaagaagaguaagaagaaauauaagagccaccaugagcucaaaggggaguguggugcuggccuauucuggcgggcuggauaccucuugcauucugguguggcugaaggaacaggguuacgacgugaucgcauaccuggccaacauugggcagaaggaggauuuugaggaagcuagaaagaaagcacugaaacucggcgccaagaaaguguucaucgaggacgucucccgggaauucguggaggaauuuaucuggccagccauucagagcuccgcucuguacgaggauagauaucugcucggaaccagccucgcacgacccugcaucgccaggaagcagguggagauugcucagcgcgaaggggcaaaguacgucucccacggugccacaggcaaaggaaacgaccaggugcgauuugagcugucuuguuauagucucgcaccccagaucaaggucauugcccccuggcgcaugcccgaguucuacaaccgguuuaagggccgcaacgaccugauggaauacgcuaaacagcacggaaucccaauucccgugacuccuaagaaccccugguccauggaugagaaucugaugcauaucucuuacgaggcugggauucucgaaaacccuaagaaucaggcacccccuggucuguauacuaagacccaggacccagccaaagcucccaacacaccugauauccuggagauugaauuuaagaaaggggugccugucaaagugacuaacgugaaagacgguaccacacaccagaccucucuggagcucuuuauguaccugaacgaagucgcaggcaagcacgggguggguagaaucgauauugucgagaaucgguucaucgggaugaaaagucgcgguauuuacgaaaccccugcuggaacaauccuguaucacgcccaucucgacauugaggcuuucacaauggauagagaagugagaaagaucaaacagggccugggacucaaguucgccgagcugguguacacuggauuuuggcacucuccagagugcgaauucgugcgacauuguaucgcuaagagucaggagagggucgaagggaagguccaggugucaguccugaaaggccagguguacauucucggacgggagucaccccugagccucuauaacgaggaacuggugagcaugaacguccagggcgacuacgaaccuacagacgccacuggauucaucaacaucaacucacucaggcucaaggaauaccacaggcuccagucaaaagucacagcaaaguaggcggccgcuuaauuaagcugccuucugcggggcuugccuucuggccaugcccuucuucucucccuugcaccuguaccucuuggucuuugaauaaagccugaguaggaag